European Patent Application EP 4 389 901 A1, published June 26, 2024. Title: 폴리 A 테일을 안정적으로 유지하는 방법. Applicant: 에스케이바이오사이언스 주식회사. The sequence listing filed with the application follows.

SEQUENCE LISTING (7 sequences)

SEQ ID NO: 1 - DNA, 164 bp, synthetic construct
  source 1..164: mol_type = other DNA
attttcattgcccgcggaaaaaaaaaaaaaaaaaaaaaaaaaaaaaaaaaaaaaaaaaaaaaaaaaaaaaaaaaaaaaaaaaaaaaaaaaaaaaaaaaaaaaaaaaaaaaaaaaaaaaaaaaaaaaaaaaaaaaaaaaaaaaagtcttcgatatcaagcttggc

SEQ ID NO: 2 - DNA, 24 bp, synthetic construct
  source 1..24: mol_type = other DNA
gccaagcttgatatcgaagacttt

SEQ ID NO: 3 - DNA, 3029 bp, synthetic construct
  source 1..3029: mol_type = other DNA
tcgcgcgtttcggtgatgacggtgaaaacctctgacacatgcagctcccggagacggtcacagcttgtctgtaagcggatgccgggagcagacaagcccgtcagggcgcgtcagcgggtgttggcgggtgtcggggctggcttaactatgcggcatcagagcagattgtactgagagtgcaccatatgcggtgtgaaataccgcacagatgcgtaaggagaaaataccgcatcaggcgccattcgccattcaggctgcgcaactgttgggaagggcgatcggtgcgggcctcttcgctattacgccagctggcgaaagggggatgtgctgcaaggcgattaagttgggtaacgccagggttttcccagtcacgacgttgtaaaacgacggccagtgaattcgagctcggtacctaatacgactcactatagggagaactcttctggtccccacagactcagagagaagccaccggatcctctagaagctcgcttgtcaatttctattaaaggttcctttgttccctaagtccaactactaaactgggggatattatgaagggccttgagcatctggattctgcctaataaaaaacatttattttcattgcatcgatagctcgctttcttgctgtccaatttctattaaaggttcctttgttccctaagtccaactactaaactgggggatattatgaagggccttgagcatctggattctgcctaataaaaaacatttattttcattgcccgcggaaaaaaaaaaaaaaaaaaaaaagtcttcgatatcaagcttggcgtaatcatggtcatagctgtttcctgtgtgaaattgttatccgctcacaattccacacaacatacgagccggaagcataaagtgtaaagcctggggtgcctaatgagtgagctaactcacattaattgcgttgcgctcactgcccgctttccagtcgggaaacctgtcgtgccagctgcattaatgaatcggccaacgcgcggggagaggcggtttgcgtattgggcgctcttccgcttcctcgctcactgactcgctgcgctcggtcgttcggctgcggcgagcggtatcagctcactcaaaggcggtaatacggttatccacagaatcaggggataacgcaggaaagaacatgtgagcaaaaggccagcaaaaggccaggaaccgtaaaaaggccgcgttgctggcgtttttccataggctccgcccccctgacgagcatcacaaaaatcgacgctcaagtcagaggtggcgaaacccgacaggactataaagataccaggcgtttccccctggaagctccctcgtgcgctctcctgttccgaccctgccgcttaccggatacctgtccgcctttctcccttcgggaagcgtggcgctttctcatagctcacgctgtaggtatctcagttcggtgtaggtcgttcgctccaagctgggctgtgtgcacgaaccccccgttcagcccgaccgctgcgccttatccggtaactatcgtcttgagtccaacccggtaagacacgacttatcgccactggcagcagccactggtaacaggattagcagagcgaggtatgtaggcggtgctacagagttcttgaagtggtggcctaactacggctacactagaagaacagtatttggtatctgcgctctgctgaagccagttaccttcggaaaaagagttggtagctcttgatccggcaaacaaaccaccgctggtagcggtggtttttttgtttgcaagcagcagattacgcgcagaaaaaaaggatctcaagaagatcctttgatcttttctacggggtctgacgctcagtggaacgaaaactcacgttaagggattttggtcatgagattatcaaaaaggatcttcacctagatccttttaaattaaaaatgaagttttaaatcaatctaaagtatatatgagtaaacttggtctgacagttaccaatgcttaatcagtgaggcacctatctcagcgatctgtctatttcgttcatccatagttgcctgactccccgtcgtgtagataactacgatacgggagggcttaccatctggccccagtgctgcaatgataccgcgagacccacgctcaccggctccagatttatcagcaataaaccagccagccggaagggccgagcgcagaagtggtcctgcaactttatccgcctccatccagtctattaattgttgccgggaagctagagtaagtagttcgccagttaatagtttgcgcaacgttgttgccattgctacaggcatcgtggtgtcacgctcgtcgtttggtatggcttcattcagctccggttcccaacgatcaaggcgagttacatgatcccccatgttgtgcaaaaaagcggttagctccttcggtcctccgatcgttgtcagaagtaagttggccgcagtgttatcactcatggttatggcagcactgcataattctcttactgtcatgccatccgtaagatgcttttctgtgactggtgagtactcaaccaagtcattctgagaatagtgtatgcggcgaccgagttgctcttgcccggcgtcaatacgggataataccgcgccacatagcagaactttaaaagtgctcatcattggaaaacgttcttcggggcgaaaactctcaaggatcttaccgctgttgagatccagttcgatgtaacccactcgtgcacccaactgatcttcagcatcttttactttcaccagcgtttctgggtgagcaaaaacaggaaggcaaaatgccgcaaaaaagggaataagggcgacacggaaatgttgaatactcatactcttcctttttcaatattattgaagcatttatcagggttattgtctcatgagcggatacatatttgaatgtatttagaaaaataaacaaataggggttccgcgcacatttccccgaaaagtgccacctgacgtctaagaaaccattattatcatgacattaacctataaaaataggcgtatcacgaggccctttcgtc

SEQ ID NO: 4 - DNA, 17 bp, synthetic construct
  source 1..17: mol_type = other DNA
gtaaaacgacggccagt

SEQ ID NO: 5 - DNA, 17 bp, synthetic construct
  source 1..17: mol_type = other DNA
caggaaacagctatgac

SEQ ID NO: 6 - DNA, 20 bp, synthetic construct
  source 1..20: mol_type = other DNA
tggataaccgtattaccgcc

SEQ ID NO: 7 - DNA, 29 bp, synthetic construct
  source 1..29: mol_type = other DNA
tcctctagaagctcgcttgtcaatttcta